European Patent Application EP 4 471 132 A1, published December 4, 2024. Title: Oncolytic virus and use thereof. Applicant: JOINT BIOSCIENCES (SH) LTD. The sequence listing filed with the application follows.

SEQUENCE LISTING (84 sequences)

SEQ ID NO: 1 - protein, 229 aa, Vesicular Stomatitis Virus
MSSLKKILGLKGKGKKSKKLGIAPPPYEEDTNMEYAPSAPIDKSYFGVNEMDTHDPNQLRYEKFFFTVKMTVRSNRPFRTYSDVAAAVSHWDHMYIGMAGKRPFYKILAFLGSSNLKATPAVLADQGQPEYHAHCEGRAYLPHRMGKTPPMLNVPEHFRRPFNIGLYKGTIELTMTIYDDESLEAAPMIWDHFNSSKFSDFREKALMFGLIVEKKASGAWVLDSVSHFK

SEQ ID NO: 2 - protein, 229 aa, (Artificial Sequence)
MSSLKKILGLKGKGKKSKKLEIAPPPYEEDTNMEYAPSAPIDKSYFGVNEMDTHDPNQLRYEKFFFTVKMTVRSNRPFRTYSDVAAAVSHWDHMYIGMAGKRPFYKILAFLGSSNLKATPAVLADQGQPEYHAHCEGRAYLPHRMGKTPPMLNVPEHFRRPFNIGLYKGTIELTMTIYDDESLEAAPMIWDHFNSSKFSDFREKALMFGLIVEKKASGAWVLDSVSHFK

SEQ ID NO: 3 - protein, 229 aa, (Artificial Sequence)
MSSLKKILGLKGKGKKSKKLEIAPPPYEEDTSMEYAPSAPIDKSYFGVNEMDTHDPNQLRYEKFFFTVKMTVRSNRPFRTYSDVAAAVSHWDHMYIGMAGKRPFYKILAFLGSSNLKATPAVLADQGQPEYHAHCEGRAYLPHRMGKTPPMLNVPEHFRRPFNIGLYKGTIELTMTIYDDESLEAAPMIWDHFNSSKFSDFREKALMFGLIVEKKASGAWVLDSVSHFK

SEQ ID NO: 4 - protein, 229 aa, (Artificial Sequence)
MSSLKKILGLKGKGKKSKKLEIAPPPYEEDTSAEYAPSAPIDKSYFGVNEMDTHDPNQLRYEKFFFTVKMTVRSNRPFRTYSDVAAAVSHWDHMYIGMAGKRPFYKILAFLGSSNLKATPAVLADQGQPEYHAHCEGRAYLPHRMGKTPPMLNVPEHFRRPFNIGLYKGTIELTMTIYDDESLEAAPMIWDHFNSSKFSDFREKALMFGLIVEKKASGAWVLDSVSHFK

SEQ ID NO: 5 - protein, 229 aa, (Artificial Sequence)
MSSLKKILGLKGKGKKSKKLEIAPPPYEEDTSAEYAPSAPIDKSYFGVDEMDTHDPNQLRYEKFFFTVKMTVRSNRPFRTYSDVAAAVSHWDHMYIGMAGKRPFYKILAFLGSSNLKATPAVLADQGQPEYHAHCEGRAYLPHRMGKTPPMLNVPEHFRRPFNIGLYKGTIELTMTIYDDESLEAAPMIWDHFNSSKFSDFREKALMFGLIVEKKASGAWVLDSVSHFK

SEQ ID NO: 6 - protein, 229 aa, (Artificial Sequence)
MSSLKKILGLKGKGKKSKKLEIAPPPYEEDTSAEYAPSAPIDKSYFGVDEMDTYDPNQLRYEKFFFTVKMTVRSNRPFRTYSDVAAAVSHWDHMYIGMAGKRPFYKILAFLGSSNLKATPAVLADQGQPEYHAHCEGRAYLPHRMGKTPPMLNVPEHFRRPFNIGLYKGTIELTMTIYDDESLEAAPMIWDHFNSSKFSDFREKALMFGLIVEKKASGAWVLDSVSHFK

SEQ ID NO: 7 - protein, 229 aa, (Artificial Sequence)
MSSLKKILGLKGKGKKSKKLEIAPPPYEEDTSAEYAPSAPIDKSYFGVDEMDTYDPNQLRYEKFFFTVKMTVRSNRPFRTYSDVAAAVSHWDHMYIGMAGKRPFYKILAFAGSSNLKATPAVLADQGQPEYHAHCEGRAYLPHRMGKTPPMLNVPEHFRRPFNIGLYKGTIELTMTIYDDESLEAAPMIWDHFNSSKFSDFREKALMFGLIVEKKASGAWVLDSVSHFK

SEQ ID NO: 8 - protein, 229 aa, (Artificial Sequence)
MSSLKKILGLKGKGKKSKKLEIAPPPYEEDTSAEYAPSAPIDKSYFGVDEMDTYDPNQLRYEKFFFTVKMTVRSNRPFRTYSDVAAAVSHWDHMYIGMAGKRPFYKILAFAGSSNLKATPAVLADQGQPEYHTHCEGRAYLPHRMGKTPPMLNVPEHFRRPFNIGLYKGTIELTMTIYDDESLEAAPMIWDHFNSSKFSDFREKALMFGLIVEKKASGAWVLDSVSHFK

SEQ ID NO: 9 - protein, 229 aa, (Artificial Sequence)
MSSLKKILGLKGKGKKSKKLEIAPPPYEEDTSAEYAPSAPIDKSYFGVDEMDTYDPNQLRYEKFFFTVKMTVRSNRPFRTYSDVAAAVSHWDHMYIGMAGKRPFYKILAFAGSSNLKATPAVLADQGQPEYHTHCEGRAYLPHRMGKTPPMLNVPEHFRRPFNIGLYKGTIELTMTIYDDESLEAAPMIWDHFNSSKFSDFREKALMFGLIVEKKASGAWVLDSISHFK

SEQ ID NO: 10 - protein, 229 aa, (Artificial Sequence)
MSSLKKILGLKGKGKKSKKLEIAPPPYEEDTSAEYAPSAPIDKSYFGVDERDTYDPNQLRYEKFFFTVKMTVRSNRPFRTYSDVAAAVSHWDHMYIGMAGKRPFYKILAFAGSSNLKATPAVLADQGQPEYHTHCEGRAYLPHRMGKTPPMLNVPEHFRRPFNIGLYKGTIELTMTIYDDESLEAAPMIWDHFNSSKFSDFREKALMFGLIVEKKASGAWVLDSISHFK

SEQ ID NO: 11 - protein, 229 aa, (Artificial Sequence)
MSSLKKILGLKGKGKKSKKLEIAPPPYEEDTSAEYAPSAPIDKSYFGVDERDTYDPNQLRYEKFFFTVKMTVRSNRPFRTYSDVAAAVSHWDHMYIGMAGKRPFYKILAFAGSSNLKATPAVLADQGQPEYHTHCEGRAYLPHRMGKTPPMLNVPEHFRRPFNIGLYKGTIELTMTIYDDESLEAAPMIWDHFNSSKFSDFREKALMFGLIVEKKASGAWFLDSISHFK

SEQ ID NO: 12 - protein, 229 aa, (Artificial Sequence)
MSSLKKILGLKGKGKKSKKLEIAPPPYEEDTSAEYAPSAPIDKSYFGVDERDTYDPNQLRYEKFFFTVKMTVRSNRPFRTYSDVAAAVSHWDHMYIGMAGKRPFYKILAFAGSSNLKATPAVLADQGQPEYHTHCEGRAYLPHRMGKTPPMLNVPEHFRRPFNIGLYKGTIELTMTIYDDESLEAAPMIWDHFNSSKFSDFREKALMFGLIVEKKASGAWFLDSIRHFK

SEQ ID NO: 13 - protein, 229 aa, (Artificial Sequence)
MSSLKKILGLKGKGKKSKKLGIAPPPYEEDTSAEYAPSAPIDKSYFGVDERDTYDPNQLRYEKFFFTVKMTVRSNRPFRTYSDVAAAVSHWDHMYIGMAGKRPFYKILAFAGSSNLKATPAVLADQGQPEYHTHCEGRAYLPHRMGKTPPMLNVPEHFRRPFNIGLYKGTIELTMTIYDDESLEAAPMIWDHFNSSKFSDFREKALMFGLIVEKKASGAWFLDSIRHFK

SEQ ID NO: 14 - protein, 229 aa, (Artificial Sequence)
MSSLKKILGLKGKGKKSKKLGIAPPPYEEDTNAEYAPSAPIDKSYFGVDERDTYDPNQLRYEKFFFTVKMTVRSNRPFRTYSDVAAAVSHWDHMYIGMAGKRPFYKILAFAGSSNLKATPAVLADQGQPEYHTHCEGRAYLPHRMGKTPPMLNVPEHFRRPFNIGLYKGTIELTMTIYDDESLEAAPMIWDHFNSSKFSDFREKALMFGLIVEKKASGAWFLDSIRHFK

SEQ ID NO: 15 - protein, 229 aa, (Artificial Sequence)
MSSLKKILGLKGKGKKSKKLGIMPPPYEEDTNAEYAPSAPIDKSYFGVDERDTYDPNQLRYEKFFFTVKMTVRSNRPFRTYSDVAAAVSHWDHMYIGMAGKRPFYKILAFAGSSNLKATPAVLADQGQPEYHTHCEGRAYLPHRMGKTPPMLNVPEHFRRPFNIGLYKGTIELTMTIYDDESLEAAPMIWDHFNSSKFSDFREKALMFGLIVEKKASGAWFLDSIRHFK

SEQ ID NO: 16 - protein, 229 aa, (Artificial Sequence)
MSSLKKILGLKGKGKKSKKLGIMPPPYEEDTNAEYAPSAPIDKSYFGVNERDTYDPNQLRYEKFFFTVKMTVRSNRPFRTYSDVAAAVSHWDHMYIGMAGKRPFYKILAFAGSSNLKATPAVLADQGQPEYHTHCEGRAYLPHRMGKTPPMLNVPEHFRRPFNIGLYKGTIELTMTIYDDESLEAAPMIWDHFNSSKFSDFREKALMFGLIVEKKASGAWFLDSIRHFK

SEQ ID NO: 17 - protein, 229 aa, (Artificial Sequence)
MSSLKKILGLKGKGKKSKKLGIMPPPYEEDTNAEYAPSAPIDKSYFGVNEMDTYDPNQLRYEKFFFTVKMTVRSNRPFRTYSDVAAAVSHWDHMYIGMAGKRPFYKILAFAGSSNLKATPAVLADQGQPEYHTHCEGRAYLPHRMGKTPPMLNVPEHFRRPFNIGLYKGTIELTMTIYDDESLEAAPMIWDHFNSSKFSDFREKALMFGLIVEKKASGAWFLDSIRHFK

SEQ ID NO: 18 - protein, 229 aa, (Artificial Sequence)
MSSLKKILGLKGKGKKSKKLGIMPPPYEEDTNAEYAPSAPIDKSYFGVNEMDTHDPNQLRYEKFFFTVKMTVRSNRPFRTYSDVAAAVSHWDHMYIGMAGKRPFYKILAFAGSSNLKATPAVLADQGQPEYHTHCEGRAYLPHRMGKTPPMLNVPEHFRRPFNIGLYKGTIELTMTIYDDESLEAAPMIWDHFNSSKFSDFREKALMFGLIVEKKASGAWFLDSIRHFK

SEQ ID NO: 19 - protein, 229 aa, (Artificial Sequence)
MSSLKKILGLKGKGKKSKKLGIMPPPYEEDTNAEYAPSAPIDKSYFGVNEMDTHDPNQLRYEKFFFTVKMTVRSNRPFRTYSDVAAAVSHWDHMYIGMAGKRPFYKILAFLGSSNLKATPAVLADQGQPEYHTHCEGRAYLPHRMGKTPPMLNVPEHFRRPFNIGLYKGTIELTMTIYDDESLEAAPMIWDHFNSSKFSDFREKALMFGLIVEKKASGAWFLDSIRHFK

SEQ ID NO: 20 - protein, 229 aa, (Artificial Sequence)
MSSLKKILGLKGKGKKSKKLGIMPPPYEEDTNAEYAPSAPIDKSYFGVNEMDTHDPNQLRYEKFFFTVKMTVRSNRPFRTYSDVAAAVSHWDHMYIGMAGKRPFYKILAFLGSSNLKATPAVLADQGQPEYHAHCEGRAYLPHRMGKTPPMLNVPEHFRRPFNIGLYKGTIELTMTIYDDESLEAAPMIWDHFNSSKFSDFREKALMFGLIVEKKASGAWFLDSIRHFK

SEQ ID NO: 21 - protein, 229 aa, (Artificial Sequence)
MSSLKKILGLKGKGKKSKKLGIMPPPYEEDTNAEYAPSAPIDKSYFGVNEMDTHDPNQLRYEKFFFTVKMTVRSNRPFRTYSDVAAAVSHWDHMYIGMAGKRPFYKILAFLGSSNLKATPAVLADQGQPEYHAHCEGRAYLPHRMGKTPPMLNVPEHFRRPFNIGLYKGTIELTMTIYDDESLEAAPMIWDHFNSSKFSDFREKALMFGLIVEKKASGAWVLDSIRHFK

SEQ ID NO: 22 - protein, 229 aa, (Artificial Sequence)
MSSLKKILGLKGKGKKSKKLGIMPPPYEEDTNAEYAPSAPIDKSYFGVNEMDTHDPNQLRYEKFFFTVKMTVRSNRPFRTYSDVAAAVSHWDHMYIGMAGKRPFYKILAFLGSSNLKATPAVLADQGQPEYHAHCEGRAYLPHRMGKTPPMLNVPEHFRRPFNIGLYKGTIELTMTIYDDESLEAAPMIWDHFNSSKFSDFREKALMFGLIVEKKASGAWVLDSVRHFK

SEQ ID NO: 23 - protein, 229 aa, (Artificial Sequence)
MSSLKKILGLKGKGKKSKKLGIAPPPYEEDTSMEYAPSAPIDKSYFGVDEMDTYDPNQLRYEKFFFTVKMTVRSNRPFRTYSDVAAAVSHWDHMYIGMAGKRPFYKILAFLGSSNLKATPAVLADQGQPEYHAHCEGRAYLPHRMGKTPPMLNVPEHFRRPFNIGLYKGTIELTMTIYDDESLEAAPMIWDHFNSSKFSDFREKALMFGLIVEKKASGAWVLDSISHFK

SEQ ID NO: 24 - protein, 229 aa, (Artificial Sequence)
MSSLKKILGLKGKGKKSKKLGIAPPPYEEDTSMEYAPSAPIDKSYFGVDEMDTYDPNQLRYEKFFFTVKMTVRSNRPFRTYSDVAAAVSHWDHMYIGMAGKRPFYKILAFLGSSNLKATPAVLADQGQPEYHAHCEGRAYLPHRMGKTPPMLNVPEHFRRPFNIGLYKGTIELTMTIYDDESLEAAPMIWDHFNSSKFSDFREKALMFGLIVEKKASGAWVLDSIGHFK

SEQ ID NO: 25 - protein, 229 aa, (Artificial Sequence)
MSSLKKILGLKGKGKKSKKLGIAPPPYEEDTSMEYAPSAPIDKSYFGVDERDTYDPNQLRYEKFFFTVKMTVRSNRPFRTYSDVAAAVSHWDHMYIGMAGKRPFYKILAFLGSSNLKATPAVLADQGQPEYHAHCEGRAYLPHRMGKTPPMLNVPEHFRRPFNIGLYKGTIELTMTIYDDESLEAAPMIWDHFNSSKFSDFREKALMFGLIVEKKASGAWFLDSIRHFK

SEQ ID NO: 26 - protein, 229 aa, (Artificial Sequence)
MSSLKKILGLKGKGKKSKKLGIAPPPYEEDTSAEYAPSAPIDKSYFGVDERDTYDPNQLRYEKFFFTVKMTVRSNRPFRTYSDVAAAVSHWDHMYIGMAGKRPFYKILAFLGSSNLKATPAVLADQGQPEYHAHCEGRAYLPHRMGKTPPMLNVPEHFRRPFNIGLYKGTIELTMTIYDDESLEAAPMIWDHFNSSKFSDFREKALMFGLIVEKKASGAWFLDSIRHFK

SEQ ID NO: 27 - protein, 229 aa, (Artificial Sequence)
MSSLKKILGLKGKGKKSKKLGIAPPPYEEDTSMEYAPSAPIDKSYFGVDERDTYDPNQLRYEKFFFTVKMTVRSNRPFRTYSDVAAAVSHWDHMYIGMAGKRPFYKILAFLGSSNLKATPAVLADQGQPEYHTHCEGRAYLPHRMGKTPPMLNVPEHFRRPFNIGLYKGTIELTMTIYDDESLEAAPMIWDHFNSSKFSDFREKALMFGLIVEKKASGAWFLDSIRHFK

SEQ ID NO: 28 - protein, 229 aa, (Artificial Sequence)
MSSLKKILGLKGKGKKSKKLGIAPPPYEEDTSAEYAPSAPIDKSYFGVDERDTYDPNQLRYEKFFFTVKMTVRSNRPFRTYSDVAAAVSHWDHMYIGMAGKRPFYKILAFLGSSNLKATPAVLADQGQPEYHTHCEGRAYLPHRMGKTPPMLNVPEHFRRPFNIGLYKGTIELTMTIYDDESLEAAPMIWDHFNSSKFSDFREKALMFGLIVEKKASGAWFLDSIRHFK

SEQ ID NO: 29 - protein, 229 aa, (Artificial Sequence)
MSSLKKILGLKGKGKKSKKLGIAPPPYEEDTSMEYAPSAPIDKSYFGVDERDTYDPNQLRYEKFFFTVKMTVRSNRPFRTYSDVAAAVSHWDHMYIGMAGKRPFYKILAFAGSSNLKATPAVLADQGQPEYHAHCEGRAYLPHRMGKTPPMLNVPEHFRRPFNIGLYKGTIELTMTIYDDESLEAAPMIWDHFNSSKFSDFREKALMFGLIVEKKASGAWVLDSIRHFK

SEQ ID NO: 30 - protein, 229 aa, (Artificial Sequence)
MSSLKKILGLKGKGKKSKKLGIAPPPYEEDTNMEYAPSAPIDKSYFGVNERDTHDPNQLRYEKFFFTVKMTVRSNRPFRTYSDVAAAVSHWDHMYIGMAGKRPFYKILAFLGSSNLKATPAVLADQGQPEYHAHCEGRAYLPHRMGKTPPMLNVPEHFRRPFNIGLYKGTIELTMTIYDDESLEAAPMIWDHFNSSKFSDFREKALMFGLIVEKKASGAWFLDSVRHFK

SEQ ID NO: 31 - protein, 511 aa, Vesicular Stomatitis Virus
MKCLLYLAFLFIGVNCKFTIVFPHNQKGNWKNVPSNYHYCPSSSDLNWHNDLVGTALQVKMPKSHKAIQADGWMCHASKWVTTCDFRWYGPKYITHSIRSFTPSVEQCKESIEQTKQGTWLNPGFPPQSCGYATVTDAEAAIVQVTPHHVLVDEYTGEWVDSQFINGKCSNDICPTVHNSTTWHSDYKVKGLCDSNLISMDITFFSEDGELSSLGKKGTGFRSNYFAYETGDKACKMQYCKHWGVRLPSGVWFEMADKDLFAAARFPECPEGSSISAPSQTSVDVSLIQDVERILDYSLCQETWSKIRAGLPISPVDLSYLAPKNPGTGPVFTIINGTLKYFETRYIRVDIAAPILSRMVGMISGTTTERVLWDDWAPYEDVEIGPNGVLRTSSGYKFPLYMIGHGMLDSDLHLSSKAQVFEHPHIQDAASQLPDGETLFFGDTGLSKNPIEFVEGWFSSWKSSIASFFFTIGLIIGLFLVLRVGIYLCIKLKHTKKRQIYTDIEMNRLGK

SEQ ID NO: 32 - protein, 511 aa, (Artificial Sequence)
MKCLLYLAFLFIGVNCKFTIVFPHNQKGNWKNVPSNYHYCPSSSDLNWHNDLIGTALQVKMPKSHKAIQADGWMCHASKWVTTCDFRWYGPKYITHSIRSFTPSVEQCKESIEQTKQGTWLNPGFPPQSCGYATVTDAEAAIVQVTPHHVLVDEYTGEWVDSQFINGKCSNDICPTVHNSTTWHSDYKVKGLCDSNLISMDITFFSEDGELSSLGKKGTGFRSNYFAYETGDKACKMQYCKHWGVRLPSGVWFEMADKDLFAAARFPECPEGSSISAPSQTSVDVSLIQDVERILDYSLCQETWSKIRAGLPISPVDLSYLAPKNPGTGPVFTIINGTLKYFETRYIRVDIAAPILSRMVGMISGTTTERVLWDDWAPYEDVEIGPNGVLRTSSGYKFPLYMIGHGMLDSDLHLSSKAQVFEHPHIQDAASQLPDGETLFFGDTGLSKNPIEFVEGWFSSWKSSIASFFFTIGLIIGLFLVLRVGIYLCIKLKHTKKRQIYTDIEMNRLGK

SEQ ID NO: 33 - protein, 511 aa, (Artificial Sequence)
MKCLLYLAFLFIGVNCKFTIVFPHNQKGNWKNVPSNYHYCPSSSDLNWHNDLIGTALQVKMPKSHKAIQADGWMCHASKWVTTCDFRWYGPKYITHSIRSFTPSVEQCKESIEQTKQGTWLNPGFPPQSCGYATVTDAEAVIVQVTPHHVLVDEYTGEWVDSQFINGKCSNDICPTVHNSTTWHSDYKVKGLCDSNLISMDITFFSEDGELSSLGKKGTGFRSNYFAYETGDKACKMQYCKHWGVRLPSGVWFEMADKDLFAAARFPECPEGSSISAPSQTSVDVSLIQDVERILDYSLCQETWSKIRAGLPISPVDLSYLAPKNPGTGPVFTIINGTLKYFETRYIRVDIAAPILSRMVGMISGTTTERVLWDDWAPYEDVEIGPNGVLRTSSGYKFPLYMIGHGMLDSDLHLSSKAQVFEHPHIQDAASQLPDGETLFFGDTGLSKNPIEFVEGWFSSWKSSIASFFFTIGLIIGLFLVLRVGIYLCIKLKHTKKRQIYTDIEMNRLGK

SEQ ID NO: 34 - protein, 511 aa, (Artificial Sequence)
MKCLLYLAFLFIGVNCKFTIVFPHNQKGNWKNVPSNYHYCPSSSDLNWHNDLIGTALQVKMPKSHKAIQADGWMCHASKWVTTCDFRWYGPKYITHSIRSFTPSVEQCKESIEQTKQGTWLNPGFPPQSCGYATVTDAEAVIVQVTPHHVLVDEYTGEWVDSQFINGKCSNYICPTVHNSTTWHSDYKVKGLCDSNLISMDITFFSEDGELSSLGKKGTGFRSNYFAYETGDKACKMQYCKHWGVRLPSGVWFEMADKDLFAAARFPECPEGSSISAPSQTSVDVSLIQDVERILDYSLCQETWSKIRAGLPISPVDLSYLAPKNPGTGPVFTIINGTLKYFETRYIRVDIAAPILSRMVGMISGTTTERVLWDDWAPYEDVEIGPNGVLRTSSGYKFPLYMIGHGMLDSDLHLSSKAQVFEHPHIQDAASQLPDGETLFFGDTGLSKNPIEFVEGWFSSWKSSIASFFFTIGLIIGLFLVLRVGIYLCIKLKHTKKRQIYTDIEMNRLGK

SEQ ID NO: 35 - protein, 511 aa, (Artificial Sequence)
MKCLLYLAFLFIGVNCKFTIVFPHNQKGNWKNVPSNYHYCPSSSDLNWHNDLIGTALQVKMPKSHKAIQADGWMCHASKWVTTCDFRWYGPKYITHSIRSFTPSVEQCKESIEQTKQGTWLNPGFPPQSCGYATVTDAEAVIVQVTPHHVLVDEYTGEWVDSQFINGKCSNYICPTVHNSTTWHSDYKVKGLCDSNLISMDITFFSEDGELSSLGKEGTGFRSNYFAYETGDKACKMQYCKHWGVRLPSGVWFEMADKDLFAAARFPECPEGSSISAPSQTSVDVSLIQDVERILDYSLCQETWSKIRAGLPISPVDLSYLAPKNPGTGPVFTIINGTLKYFETRYIRVDIAAPILSRMVGMISGTTTERVLWDDWAPYEDVEIGPNGVLRTSSGYKFPLYMIGHGMLDSDLHLSSKAQVFEHPHIQDAASQLPDGETLFFGDTGLSKNPIEFVEGWFSSWKSSIASFFFTIGLIIGLFLVLRVGIYLCIKLKHTKKRQIYTDIEMNRLGK

SEQ ID NO: 36 - protein, 511 aa, (Artificial Sequence)
MKCLLYLAFLFIGVNCKFTIVFPHNQKGNWKNVPSNYHYCPSSSDLNWHNDLIGTALQVKMPKSHKAIQADGWMCHASKWVTTCDFRWYGPKYITHSIRSFTPSVEQCKESIEQTKQGTWLNPGFPPQSCGYATVTDAEAVIVQVTPHHVLVDEYTGEWVDSQFINGKCSNYICPTVHNSTTWHSDYKVKGLCDSNLISMDITFFSEDGELSSLGKEGTGFRSNYFAYETGGKACKMQYCKHWGVRLPSGVWFEMADKDLFAAARFPECPEGSSISAPSQTSVDVSLIQDVERILDYSLCQETWSKIRAGLPISPVDLSYLAPKNPGTGPVFTIINGTLKYFETRYIRVDIAAPILSRMVGMISGTTTERVLWDDWAPYEDVEIGPNGVLRTSSGYKFPLYMIGHGMLDSDLHLSSKAQVFEHPHIQDAASQLPDGETLFFGDTGLSKNPIEFVEGWFSSWKSSIASFFFTIGLIIGLFLVLRVGIYLCIKLKHTKKRQIYTDIEMNRLGK

SEQ ID NO: 37 - protein, 511 aa, (Artificial Sequence)
MKCLLYLAFLFIGVNCKFTIVFPHNQKGNWKNVPSNYHYCPSSSDLNWHNDLIGTALQVKMPKSHKAIQADGWMCHASKWVTTCDFRWYGPKYITHSIRSFTPSVEQCKESIEQTKQGTWLNPGFPPQSCGYATVTDAEAVIVQVTPHHVLVDEYTGEWVDSQFINGKCSNYICPTVHNSTTWHSDYKVKGLCDSNLISMDITFFSEDGELSSLGKEGTGFRSNYFAYETGGKACKMQYCKHWGVRLPSGVWFEMADKDLFAAARFPECPEGSSISAPSQTSVDVSLIQDVERILDYSLCQETWSKIRAGLPISPVDLSYLAPKNPGTGPAFTIINGTLKYFETRYIRVDIAAPILSRMVGMISGTTTERVLWDDWAPYEDVEIGPNGVLRTSSGYKFPLYMIGHGMLDSDLHLSSKAQVFEHPHIQDAASQLPDGETLFFGDTGLSKNPIEFVEGWFSSWKSSIASFFFTIGLIIGLFLVLRVGIYLCIKLKHTKKRQIYTDIEMNRLGK

SEQ ID NO: 38 - protein, 511 aa, (Artificial Sequence)
MKCLLYLAFLFIGVNCKFTIVFPHNQKGNWKNVPSNYHYCPSSSDLNWHNDLIGTALQVKMPKSHKAIQADGWMCHASKWVTTCDFRWYGPKYITHSIRSFTPSVEQCKESIEQTKQGTWLNPGFPPQSCGYATVTDAEAVIVQVTPHHVLVDEYTGEWVDSQFINGKCSNYICPTVHNSTTWHSDYKVKGLCDSNLISMDITFFSEDGELSSLGKEGTGFRSNYFAYETGGKACKMQYCKHWGVRLPSGVWFEMADKDLFAAARFPECPEGSSISAPSQTSVDVSLIQDVERILDYSLCQETWSKIRAGLPISPVDLSYLAPKNPGTGPAFTIINGTLKYFETRYIRVDIAAPILSRMVGMISGTTTERELWDDWAPYEDVEIGPNGVLRTSSGYKFPLYMIGHGMLDSDLHLSSKAQVFEHPHIQDAASQLPDGETLFFGDTGLSKNPIEFVEGWFSSWKSSIASFFFTIGLIIGLFLVLRVGIYLCIKLKHTKKRQIYTDIEMNRLGK

SEQ ID NO: 39 - protein, 511 aa, (Artificial Sequence)
MKCLLYLAFLFIGVNCKFTIVFPHNQKGNWKNVPSNYHYCPSSSDLNWHNDLIGTALQVKMPKSHKAIQADGWMCHASKWVTTCDFRWYGPKYITHSIRSFTPSVEQCKESIEQTKQGTWLNPGFPPQSCGYATVTDAEAVIVQVTPHHVLVDEYTGEWVDSQFINGKCSNYICPTVHNSTTWHSDYKVKGLCDSNLISMDITFFSEDGELSSLGKEGTGFRSNYFAYETGGKACKMQYCKHWGVRLPSGVWFEMADKDLFAAARFPECPEGSSISAPSQTSVDVSLIQDVERILDYSLCQETWSKIRAGLPISPVDLSYLAPKNPGTGPAFTIINGTLKYFETRYIRVDIAAPILSRMVGMISGTTTERELWDDWAPYEDVEIGPNGVLRTSSGYKFPLYMIGHGMLDSDLHLSSKAQVFEHPHIQDAASQLPDDETLFFGDTGLSKNPIEFVEGWFSSWKSSIASFFFTIGLIIGLFLVLRVGIYLCIKLKHTKKRQIYTDIEMNRLGK

SEQ ID NO: 40 - protein, 511 aa, (Artificial Sequence)
MKCLLYLAFLFIGVNCKFTIVFPHNQKGNWKNVPSNYHYCPSSSDLNWHNDLIGTALQVKMPKSHKAIQADGWMCHASKWVTTCDFRWYGPKYITHSIRSFTPSVEQCKESIEQTKQGTWLNPGFPPQSCGYATVTDAEAVIVQVTPHHVLVDEYTGEWVDSQFINGKCSNYICPTVHNSTTWHSDYKVKGLCDSNLISMDITFFSEDGELSSLGKEGTGFRSNYFAYETGGKACKMQYCKHWGVRLPSGVWFEMADKDLFAAARFPECPEGSSISAPSQTSVDVSLIQDVERILDYSLCQETWSKIRAGLPISPVDLSYLAPKNPGTGPAFTIINGTLKYFETRYIRVDIAAPILSRMVGMISGTTTERELWDDWAPYEDVEIGPNGVLRTSSGYKFPLYMIGHGMLDSDLHLSSKAQVFEHPHIQDAASQLPDDESLFFGDTGLSKNPIEFVEGWFSSWKSSIASFFFTIGLIIGLFLVLRVGIYLCIKLKHTKKRQIYTDIEMNRLGK

SEQ ID NO: 41 - protein, 511 aa, (Artificial Sequence)
MKCLLYLAFLFIGVNCKFTIVFPHNQKGNWKNVPSNYHYCPSSSDLNWHNDLIGTALQVKMPKSHKAIQADGWMCHASKWVTTCDFRWYGPKYITHSIRSFTPSVEQCKESIEQTKQGTWLNPGFPPQSCGYATVTDAEAVIVQVTPHHVLVDEYTGEWVDSQFINGKCSNYICPTVHNSTTWHSDYKVKGLCDSNLISMDITFFSEDGELSSLGKEGTGFRSNYFAYETGGKACKMQYCKHWGVRLPSGVWFEMADKDLFAAARFPECPEGSSISAPSQTSVDVSLIQDVERILDYSLCQETWSKIRAGLPISPVDLSYLAPKNPGTGPAFTIINGTLKYFETRYIRVDIAAPILSRMVGMISGTTTERELWDDWAPYEDVEIGPNGVLRTSSGYKFPLYMIGHGMLDSDLHLSSKAQVFEHPHIQDAASQLPDDESLFFGDTGLSKNPIELVEGWFSSWKSSIASFFFTIGLIIGLFLVLRVGIYLCIKLKHTKKRQIYTDIEMNRLGK

SEQ ID NO: 42 - protein, 511 aa, (Artificial Sequence)
MKCLLYLAFLFIGVNCKFTIVFPHNQKGNWKNVPSNYHYCPSSSDLNWHNDLIGTALQVKMPKSHKAIQADGWMCHASKWVTTCDFRWYGPKYITHSIRSFTPSVEQCKESIEQTKQGTWLNPGFPPQSCGYATVTDAEAVIVQVTPHHVLVDEYTGEWVDSQFINGKCSNYICPTVHNSTTWHSDYKVKGLCDSNLISMDITFFSEDGELSSLGKEGTGFRSNYFAYETGGKACKMQYCKHWGVRLPSGVWFEMADKDLFAAARFPECPEGSSISAPSQTSVDVSLIQDVERILDYSLCQETWSKIRAGLPISPVDLSYLAPKNPGTGPAFTIINGTLKYFETRYIRVDIAAPILSRMVGMISGTTTERELWDDWAPYEDVEIGPNGVLRTSSGYKFPLYMIGHGMLDSDLHLSSKAQVFEHPHIQDAASQLPDDESLFFGDTGLSKNPIELVEGWFSSWKSSIASFFFIIGLIIGLFLVLRVGIYLCIKLKHTKKRQIYTDIEMNRLGK

SEQ ID NO: 43 - protein, 511 aa, (Artificial Sequence)
MKCLLYLAFLFIGVNCKFTIVFPHNQKGNWKNVPSNYHYCPSSSDLNWHNDLIGTALQVKMPKSHKAIQADGWMCHASKWVTTCDFRWYGPKYITHSIRSFTPSVEQCKESIEQTKQGTWLNPGFPPQSCGYATVTDAEAVIVQVTPHHVLVDEYTGEWVDSQFINGKCSNYICPTVHNSTTWHSDYKVKGLCDSNLISMDITFFSEDGELSSLGKEGTGFRSNYFAYETGGKACKMQYCKHWGVRLPSGVWFEMADKDLFAAARFPECPEGSSISAPSQTSVDVSLIQDVERILDYSLCQETWSKIRAGLPISPVDLSYLAPKNPGTGPAFTIINGTLKYFETRYIRVDIAAPILSRMVGMISGTTTERELWDDWAPYEDVEIGPNGVLRTSSGYKFPLYMIGHGMLDSDLHLSSKAQVFEHPHIQDAASQLPDDESLFFGDTGLSKNPIELVEGWFSSWKSSIASFFFIIGLIIGLFLVLRVGIHLCIKLKHTKKRQIYTDIEMNRLGK

SEQ ID NO: 44 - protein, 511 aa, (Artificial Sequence)
MKCLLYLAFLFIGVNCKFTIVFPHNQKGNWKNVPSNYHYCPSSSDLNWHNDLVGTALQVKMPKSHKAIQADGWMCHASKWVTTCDFRWYGPKYITHSIRSFTPSVEQCKESIEQTKQGTWLNPGFPPQSCGYATVTDAEAVIVQVTPHHVLVDEYTGEWVDSQFINGKCSNYICPTVHNSTTWHSDYKVKGLCDSNLISMDITFFSEDGELSSLGKEGTGFRSNYFAYETGGKACKMQYCKHWGVRLPSGVWFEMADKDLFAAARFPECPEGSSISAPSQTSVDVSLIQDVERILDYSLCQETWSKIRAGLPISPVDLSYLAPKNPGTGPAFTIINGTLKYFETRYIRVDIAAPILSRMVGMISGTTTERELWDDWAPYEDVEIGPNGVLRTSSGYKFPLYMIGHGMLDSDLHLSSKAQVFEHPHIQDAASQLPDDESLFFGDTGLSKNPIELVEGWFSSWKSSIASFFFIIGLIIGLFLVLRVGIHLCIKLKHTKKRQIYTDIEMNRLGK

SEQ ID NO: 45 - protein, 511 aa, (Artificial Sequence)
MKCLLYLAFLFIGVNCKFTIVFPHNQKGNWKNVPSNYHYCPSSSDLNWHNDLVGTALQVKMPKSHKAIQADGWMCHASKWVTTCDFRWYGPKYITHSIRSFTPSVEQCKESIEQTKQGTWLNPGFPPQSCGYATVTDAEAAIVQVTPHHVLVDEYTGEWVDSQFINGKCSNYICPTVHNSTTWHSDYKVKGLCDSNLISMDITFFSEDGELSSLGKEGTGFRSNYFAYETGGKACKMQYCKHWGVRLPSGVWFEMADKDLFAAARFPECPEGSSISAPSQTSVDVSLIQDVERILDYSLCQETWSKIRAGLPISPVDLSYLAPKNPGTGPAFTIINGTLKYFETRYIRVDIAAPILSRMVGMISGTTTERELWDDWAPYEDVEIGPNGVLRTSSGYKFPLYMIGHGMLDSDLHLSSKAQVFEHPHIQDAASQLPDDESLFFGDTGLSKNPIELVEGWFSSWKSSIASFFFIIGLIIGLFLVLRVGIHLCIKLKHTKKRQIYTDIEMNRLGK

SEQ ID NO: 46 - protein, 511 aa, (Artificial Sequence)
MKCLLYLAFLFIGVNCKFTIVFPHNQKGNWKNVPSNYHYCPSSSDLNWHNDLVGTALQVKMPKSHKAIQADGWMCHASKWVTTCDFRWYGPKYITHSIRSFTPSVEQCKESIEQTKQGTWLNPGFPPQSCGYATVTDAEAAIVQVTPHHVLVDEYTGEWVDSQFINGKCSNDICPTVHNSTTWHSDYKVKGLCDSNLISMDITFFSEDGELSSLGKEGTGFRSNYFAYETGGKACKMQYCKHWGVRLPSGVWFEMADKDLFAAARFPECPEGSSISAPSQTSVDVSLIQDVERILDYSLCQETWSKIRAGLPISPVDLSYLAPKNPGTGPAFTIINGTLKYFETRYIRVDIAAPILSRMVGMISGTTTERELWDDWAPYEDVEIGPNGVLRTSSGYKFPLYMIGHGMLDSDLHLSSKAQVFEHPHIQDAASQLPDDESLFFGDTGLSKNPIELVEGWFSSWKSSIASFFFIIGLIIGLFLVLRVGIHLCIKLKHTKKRQIYTDIEMNRLGK

SEQ ID NO: 47 - protein, 511 aa, (Artificial Sequence)
MKCLLYLAFLFIGVNCKFTIVFPHNQKGNWKNVPSNYHYCPSSSDLNWHNDLVGTALQVKMPKSHKAIQADGWMCHASKWVTTCDFRWYGPKYITHSIRSFTPSVEQCKESIEQTKQGTWLNPGFPPQSCGYATVTDAEAAIVQVTPHHVLVDEYTGEWVDSQFINGKCSNDICPTVHNSTTWHSDYKVKGLCDSNLISMDITFFSEDGELSSLGKKGTGFRSNYFAYETGGKACKMQYCKHWGVRLPSGVWFEMADKDLFAAARFPECPEGSSISAPSQTSVDVSLIQDVERILDYSLCQETWSKIRAGLPISPVDLSYLAPKNPGTGPAFTIINGTLKYFETRYIRVDIAAPILSRMVGMISGTTTERELWDDWAPYEDVEIGPNGVLRTSSGYKFPLYMIGHGMLDSDLHLSSKAQVFEHPHIQDAASQLPDDESLFFGDTGLSKNPIELVEGWFSSWKSSIASFFFIIGLIIGLFLVLRVGIHLCIKLKHTKKRQIYTDIEMNRLGK

SEQ ID NO: 48 - protein, 511 aa, (Artificial Sequence)
MKCLLYLAFLFIGVNCKFTIVFPHNQKGNWKNVPSNYHYCPSSSDLNWHNDLVGTALQVKMPKSHKAIQADGWMCHASKWVTTCDFRWYGPKYITHSIRSFTPSVEQCKESIEQTKQGTWLNPGFPPQSCGYATVTDAEAAIVQVTPHHVLVDEYTGEWVDSQFINGKCSNDICPTVHNSTTWHSDYKVKGLCDSNLISMDITFFSEDGELSSLGKKGTGFRSNYFAYETGDKACKMQYCKHWGVRLPSGVWFEMADKDLFAAARFPECPEGSSISAPSQTSVDVSLIQDVERILDYSLCQETWSKIRAGLPISPVDLSYLAPKNPGTGPAFTIINGTLKYFETRYIRVDIAAPILSRMVGMISGTTTERELWDDWAPYEDVEIGPNGVLRTSSGYKFPLYMIGHGMLDSDLHLSSKAQVFEHPHIQDAASQLPDDESLFFGDTGLSKNPIELVEGWFSSWKSSIASFFFIIGLIIGLFLVLRVGIHLCIKLKHTKKRQIYTDIEMNRLGK

SEQ ID NO: 49 - protein, 511 aa, (Artificial Sequence)
MKCLLYLAFLFIGVNCKFTIVFPHNQKGNWKNVPSNYHYCPSSSDLNWHNDLVGTALQVKMPKSHKAIQADGWMCHASKWVTTCDFRWYGPKYITHSIRSFTPSVEQCKESIEQTKQGTWLNPGFPPQSCGYATVTDAEAAIVQVTPHHVLVDEYTGEWVDSQFINGKCSNDICPTVHNSTTWHSDYKVKGLCDSNLISMDITFFSEDGELSSLGKKGTGFRSNYFAYETGDKACKMQYCKHWGVRLPSGVWFEMADKDLFAAARFPECPEGSSISAPSQTSVDVSLIQDVERILDYSLCQETWSKIRAGLPISPVDLSYLAPKNPGTGPVFTIINGTLKYFETRYIRVDIAAPILSRMVGMISGTTTERELWDDWAPYEDVEIGPNGVLRTSSGYKFPLYMIGHGMLDSDLHLSSKAQVFEHPHIQDAASQLPDDESLFFGDTGLSKNPIELVEGWFSSWKSSIASFFFIIGLIIGLFLVLRVGIHLCIKLKHTKKRQIYTDIEMNRLGK

SEQ ID NO: 50 - protein, 511 aa, (Artificial Sequence)
MKCLLYLAFLFIGVNCKFTIVFPHNQKGNWKNVPSNYHYCPSSSDLNWHNDLVGTALQVKMPKSHKAIQADGWMCHASKWVTTCDFRWYGPKYITHSIRSFTPSVEQCKESIEQTKQGTWLNPGFPPQSCGYATVTDAEAAIVQVTPHHVLVDEYTGEWVDSQFINGKCSNDICPTVHNSTTWHSDYKVKGLCDSNLISMDITFFSEDGELSSLGKKGTGFRSNYFAYETGDKACKMQYCKHWGVRLPSGVWFEMADKDLFAAARFPECPEGSSISAPSQTSVDVSLIQDVERILDYSLCQETWSKIRAGLPISPVDLSYLAPKNPGTGPVFTIINGTLKYFETRYIRVDIAAPILSRMVGMISGTTTERVLWDDWAPYEDVEIGPNGVLRTSSGYKFPLYMIGHGMLDSDLHLSSKAQVFEHPHIQDAASQLPDDESLFFGDTGLSKNPIELVEGWFSSWKSSIASFFFIIGLIIGLFLVLRVGIHLCIKLKHTKKRQIYTDIEMNRLGK

SEQ ID NO: 51 - protein, 511 aa, (Artificial Sequence)
MKCLLYLAFLFIGVNCKFTIVFPHNQKGNWKNVPSNYHYCPSSSDLNWHNDLVGTALQVKMPKSHKAIQADGWMCHASKWVTTCDFRWYGPKYITHSIRSFTPSVEQCKESIEQTKQGTWLNPGFPPQSCGYATVTDAEAAIVQVTPHHVLVDEYTGEWVDSQFINGKCSNDICPTVHNSTTWHSDYKVKGLCDSNLISMDITFFSEDGELSSLGKKGTGFRSNYFAYETGDKACKMQYCKHWGVRLPSGVWFEMADKDLFAAARFPECPEGSSISAPSQTSVDVSLIQDVERILDYSLCQETWSKIRAGLPISPVDLSYLAPKNPGTGPVFTIINGTLKYFETRYIRVDIAAPILSRMVGMISGTTTERVLWDDWAPYEDVEIGPNGVLRTSSGYKFPLYMIGHGMLDSDLHLSSKAQVFEHPHIQDAASQLPDGESLFFGDTGLSKNPIELVEGWFSSWKSSIASFFFIIGLIIGLFLVLRVGIHLCIKLKHTKKRQIYTDIEMNRLGK

SEQ ID NO: 52 - protein, 511 aa, (Artificial Sequence)
MKCLLYLAFLFIGVNCKFTIVFPHNQKGNWKNVPSNYHYCPSSSDLNWHNDLVGTALQVKMPKSHKAIQADGWMCHASKWVTTCDFRWYGPKYITHSIRSFTPSVEQCKESIEQTKQGTWLNPGFPPQSCGYATVTDAEAAIVQVTPHHVLVDEYTGEWVDSQFINGKCSNDICPTVHNSTTWHSDYKVKGLCDSNLISMDITFFSEDGELSSLGKKGTGFRSNYFAYETGDKACKMQYCKHWGVRLPSGVWFEMADKDLFAAARFPECPEGSSISAPSQTSVDVSLIQDVERILDYSLCQETWSKIRAGLPISPVDLSYLAPKNPGTGPVFTIINGTLKYFETRYIRVDIAAPILSRMVGMISGTTTERVLWDDWAPYEDVEIGPNGVLRTSSGYKFPLYMIGHGMLDSDLHLSSKAQVFEHPHIQDAASQLPDGETLFFGDTGLSKNPIELVEGWFSSWKSSIASFFFIIGLIIGLFLVLRVGIHLCIKLKHTKKRQIYTDIEMNRLGK

SEQ ID NO: 53 - protein, 511 aa, (Artificial Sequence)
MKCLLYLAFLFIGVNCKFTIVFPHNQKGNWKNVPSNYHYCPSSSDLNWHNDLVGTALQVKMPKSHKAIQADGWMCHASKWVTTCDFRWYGPKYITHSIRSFTPSVEQCKESIEQTKQGTWLNPGFPPQSCGYATVTDAEAAIVQVTPHHVLVDEYTGEWVDSQFINGKCSNDICPTVHNSTTWHSDYKVKGLCDSNLISMDITFFSEDGELSSLGKKGTGFRSNYFAYETGDKACKMQYCKHWGVRLPSGVWFEMADKDLFAAARFPECPEGSSISAPSQTSVDVSLIQDVERILDYSLCQETWSKIRAGLPISPVDLSYLAPKNPGTGPVFTIINGTLKYFETRYIRVDIAAPILSRMVGMISGTTTERVLWDDWAPYEDVEIGPNGVLRTSSGYKFPLYMIGHGMLDSDLHLSSKAQVFEHPHIQDAASQLPDGETLFFGDTGLSKNPIEFVEGWFSSWKSSIASFFFIIGLIIGLFLVLRVGIHLCIKLKHTKKRQIYTDIEMNRLGK

SEQ ID NO: 54 - protein, 511 aa, (Artificial Sequence)
MKCLLYLAFLFIGVNCKFTIVFPHNQKGNWKNVPSNYHYCPSSSDLNWHNDLVGTALQVKMPKSHKAIQADGWMCHASKWVTTCDFRWYGPKYITHSIRSFTPSVEQCKESIEQTKQGTWLNPGFPPQSCGYATVTDAEAAIVQVTPHHVLVDEYTGEWVDSQFINGKCSNDICPTVHNSTTWHSDYKVKGLCDSNLISMDITFFSEDGELSSLGKKGTGFRSNYFAYETGDKACKMQYCKHWGVRLPSGVWFEMADKDLFAAARFPECPEGSSISAPSQTSVDVSLIQDVERILDYSLCQETWSKIRAGLPISPVDLSYLAPKNPGTGPVFTIINGTLKYFETRYIRVDIAAPILSRMVGMISGTTTERVLWDDWAPYEDVEIGPNGVLRTSSGYKFPLYMIGHGMLDSDLHLSSKAQVFEHPHIQDAASQLPDGETLFFGDTGLSKNPIEFVEGWFSSWKSSIASFFFTIGLIIGLFLVLRVGIHLCIKLKHTKKRQIYTDIEMNRLGK

SEQ ID NO: 55 - protein, 422 aa, Vesicular Stomatitis Virus
MSVTVKRIIDNTVIVPKLPANEDPVEYPADYFRKSKEIPLYINTTKSLSDLRGYVYQGLKSGNVSIIHVNSYLYGALKDIRGKLDKDWSSFGINIGKAGDTIGIFDLVSLKALDGVLPDGVSDASRTSADDKWLPLYLLGLYRVGRTQMPEYRKRLMDGLTNQCKMINEQFEPLVPEGRDIFDVWGNDSNYTKIVAAVDMFFHMFKKHECASFRYGTIVSRFKDCAALATFGHLCKITGMSTEDVTTWILNREVADEMVQMMLPGQEIDKADSYMPYLIDFGLSSKSPYSSVKNPAFHFWGQLTALLLRSTRARNARQPDDIEYTSLTTAGLLYAYAVGSSADLAQQFCVGDSKYTPDDSTGGLTTNAPPQGRDVVEWLGWFEDQNRKPTPDMMQYAKRAVMSLQGLREKTIGKYAKSEFDK

SEQ ID NO: 56 - protein, 422 aa, (Artificial Sequence)
MSVTVKRIIDNTVVVPKLPANEDPVEYPADYFRKSKEIPLYINTTKSLSDLRGYVYQGLKSGNVSIIHVNSYLYGALKDIRGKLDKDWSSFGINIGKAGDTIGIFDLVSLKALDGVLPDGVSDASRTSADDKWLPLYLLGLYRVGRTQMPEYRKRLMDGLTNQCKMINEQFEPLVPEGRDIFDVWGNDSNYTKIVAAVDMFFHMFKKHECASFRYGTIVSRFKDCAALATFGHLCKITGMSTEDVTTWILNREVADEMVQMMLPGQEIDKADSYMPYLIDFGLSSKSPYSSVKNPAFHFWGQLTALLLRSTRARNARQPDDIEYTSLTTAGLLYAYAVGSSADLAQQFCVGDSKYTPDDSTGGLTTNAPPQGRDVVEWLGWFEDQNRKPTPDMMQYAKRAVMSLQGLREKTIGKYAKSEFDK

SEQ ID NO: 57 - protein, 422 aa, (Artificial Sequence)
MSVTVKRIIDNTVVVPKLPANEDPVEYPADYFRKSKEIPLYINTTKSLSDLRGYVYQGLKSGNVSIIHVNSYLYGALKDIRGKLDKDWSSFGINIGKAGDTIGIFDLVSLKALDGVLPDGVSDASRTSADDKWLPLYLLGLYRVGRTQMPEYRKKLMDGLTNQCKMINEQFEPLVPEGRDIFDVWGNDSNYTKIVAAVDMFFHMFKKHECASFRYGTIVSRFKDCAALATFGHLCKITGMSTEDVTTWILNREVADEMVQMMLPGQEIDKADSYMPYLIDFGLSSKSPYSSVKNPAFHFWGQLTALLLRSTRARNARQPDDIEYTSLTTAGLLYAYAVGSSADLAQQFCVGDSKYTPDDSTGGLTTNAPPQGRDVVEWLGWFEDQNRKPTPDMMQYAKRAVMSLQGLREKTIGKYAKSEFDK

SEQ ID NO: 58 - protein, 422 aa, (Artificial Sequence)
MSVTVKRIIDNTVVVPKLPANEDPVEYPADYFRKSKEIPLYINTTKSLSDLRGYVYQGLKSGNVSIIHVNSYLYGALKDIRGKLDKDWSSFGINIGKAGDTIGIFDLVSLKALDGVLPDGVSDASRTSADDKWLPLYLLGLYRVGRTQMPEYRKKLMDGLTNQCKMINEQFEPLVPEGRDIFDVWGNDSNYTKIVAAVDMFFHMFKKHECASFRYGTIVSRFKDCAALATFGHLCKITGMSTEDVTTWILNREVADEMVQMMLPGQEIDKADSYMPYLIDFGLSSKSPYSSVKNPAFHFWGQLTALLLRSTRARNARQPDDIEYTSLTTAGLLYAYAVGSSADLAQQFCVGDNKYTPDDSTGGLTTNAPPQGRDVVEWLGWFEDQNRKPTPDMMQYAKRAVMSLQGLREKTIGKYAKSEFDK

SEQ ID NO: 59 - protein, 422 aa, (Artificial Sequence)
MSVTVKRIIDNTVIVPKLPANEDPVEYPADYFRKSKEIPLYINTTKSLSDLRGYVYQGLKSGNVSIIHVNSYLYGALKDIRGKLDKDWSSFGINIGKAGDTIGIFDLVSLKALDGVLPDGVSDASRTSADDKWLPLYLLGLYRVGRTQMPEYRKKLMDGLTNQCKMINEQFEPLVPEGRDIFDVWGNDSNYTKIVAAVDMFFHMFKKHECASFRYGTIVSRFKDCAALATFGHLCKITGMSTEDVTTWILNREVADEMVQMMLPGQEIDKADSYMPYLIDFGLSSKSPYSSVKNPAFHFWGQLTALLLRSTRARNARQPDDIEYTSLTTAGLLYAYAVGSSADLAQQFCVGDNKYTPDDSTGGLTTNAPPQGRDVVEWLGWFEDQNRKPTPDMMQYAKRAVMSLQGLREKTIGKYAKSEFDK

SEQ ID NO: 60 - protein, 422 aa, (Artificial Sequence)
MSVTVKRIIDNTVIVPKLPANEDPVEYPADYFRKSKEIPLYINTTKSLSDLRGYVYQGLKSGNVSIIHVNSYLYGALKDIRGKLDKDWSSFGINIGKAGDTIGIFDLVSLKALDGVLPDGVSDASRTSADDKWLPLYLLGLYRVGRTQMPEYRKRLMDGLTNQCKMINEQFEPLVPEGRDIFDVWGNDSNYTKIVAAVDMFFHMFKKHECASFRYGTIVSRFKDCAALATFGHLCKITGMSTEDVTTWILNREVADEMVQMMLPGQEIDKADSYMPYLIDFGLSSKSPYSSVKNPAFHFWGQLTALLLRSTRARNARQPDDIEYTSLTTAGLLYAYAVGSSADLAQQFCVGDNKYTPDDSTGGLTTNAPPQGRDVVEWLGWFEDQNRKPTPDMMQYAKRAVMSLQGLREKTIGKYAKSEFDK

SEQ ID NO: 61 - protein, 265 aa, Vesicular Stomatitis Virus
MDNLTKVREYLKSYSRLDQAVGEIDEIEAQRAEKSNYELFQEDGVEEHTRPSYFQAADDSDTESEPEIEDNQGLYVPDPEAEQVEGFIQGPLDDYADEDVDVVFTSDWKQPELESDEHGKTLRLTLPEGLSGEQKSQWLLTIKAVVQSAKHWNLAECTFEASGEGVIIKKRQITPDVYKVTPVMNTHPYQSEAVSDVWSLSKTSMTFQPKKASLQPLTISLDELFSSRGEFISVGGNGRMSHKEAILLGLRYKKLYNQARVKYSL

SEQ ID NO: 62 - protein, 265 aa, (Artificial Sequence)
MDNLTKVREYLKSYSRLDQAVGEIDEIEAQRAEKSNYELFQEDGVEEHTKPSYFQAADDSDTESEPEIEDNQGLYVPDPEAEQVEGFIQGPLDDYADEDVDVVFTSDWKQPELESDEHGKTLRLTLPEGLSGEQKSQWLLTIKAVVQSAKHWNLAECTFEASGEGVIIKKRQITPDVYKVTPVMNTHPYQSEAVSDVWSLSKTSMTFQPKKASLQPLTISLDELFSSRGEFISVGGNGRMSHKEAILLGLRYKKLYNQARVKYSL

SEQ ID NO: 63 - protein, 265 aa, (Artificial Sequence)
MDNLTKVREYLKSYSRLDQAVGEIDEIEAQRAEKSNYELFQEDGVEEHTKPSYFQAADDSDTESEPEIEDNQGLYAPDPEAEQVEGFIQGPLDDYADEDVDVVFTSDWKQPELESDEHGKTLRLTLPEGLSGEQKSQWLLTIKAVVQSAKHWNLAECTFEASGEGVIIKKRQITPDVYKVTPVMNTHPYQSEAVSDVWSLSKTSMTFQPKKASLQPLTISLDELFSSRGEFISVGGNGRMSHKEAILLGLRYKKLYNQARVKYSL

SEQ ID NO: 64 - protein, 265 aa, (Artificial Sequence)
MDNLTKVREYLKSYSRLDQAVGEIDEIEAQRAEKSNYELFQEDGVEEHTKPSYFQAADDSDTESEPEIEDNQGLYAPDPEAEQVEGFIQGPLDDYADEEVDVVFTSDWKQPELESDEHGKTLRLTLPEGLSGEQKSQWLLTIKAVVQSAKHWNLAECTFEASGEGVIIKKRQITPDVYKVTPVMNTHPYQSEAVSDVWSLSKTSMTFQPKKASLQPLTISLDELFSSRGEFISVGGNGRMSHKEAILLGLRYKKLYNQARVKYSL

SEQ ID NO: 65 - protein, 265 aa, (Artificial Sequence)
MDNLTKVREYLKSYSRLDQAVGEIDEIEAQRAEKSNYELFQEDGVEEHTKPSYFQAADDSDTESEPEIEDNQGLYAPDPEAEQVEGFIQGPLDDYADEEVDVVFTSDWKQPELESDEHGKTLRLTSPEGLSGEQKSQWLLTIKAVVQSAKHWNLAECTFEASGEGVIIKKRQITPDVYKVTPVMNTHPYQSEAVSDVWSLSKTSMTFQPKKASLQPLTISLDELFSSRGEFISVGGNGRMSHKEAILLGLRYKKLYNQARVKYSL

SEQ ID NO: 66 - protein, 265 aa, (Artificial Sequence)
MDNLTKVREYLKSYSRLDQAVGEIDEIEAQRAEKSNYELFQEDGVEEHTKPSYFQAADDSDTESEPEIEDNQGLYAPDPEAEQVEGFIQGPLDDYADEEVDVVFTSDWKQPELESDEHGKTLRLTSPEGLSGEQKSQWLSTIKAVVQSAKHWNLAECTFEASGEGVIIKKRQITPDVYKVTPVMNTHPYQSEAVSDVWSLSKTSMTFQPKKASLQPLTISLDELFSSRGEFISVGGNGRMSHKEAILLGLRYKKLYNQARVKYSL

SEQ ID NO: 67 - protein, 265 aa, (Artificial Sequence)
MDNLTKVREYLKSYSRLDQAVGEIDEIEAQRAEKSNYELFQEDGVEEHTKPSYFQAADDSDTESEPEIEDNQGLYAPDPEAEQVEGFIQGPLDDYADEEVDVVFTSDWKQPELESDEHGKTLRLTSPEGLSGEQKSQWLSTIKAVVQSAKYWNLAECTFEASGEGVIIKKRQITPDVYKVTPVMNTHPYQSEAVSDVWSLSKTSMTFQPKKASLQPLTISLDELFSSRGEFISVGGNGRMSHKEAILLGLRYKKLYNQARVKYSL

SEQ ID NO: 68 - protein, 265 aa, (Artificial Sequence)
MDNLTKVREYLKSYSRLDQAVGEIDEIEAQRAEKSNYELFQEDGVEEHTKPSYFQAADDSDTESEPEIEDNQGLYAPDPEAEQVEGFIQGPLDDYADEEVDVVFTSDWKQPELESDEHGKTLRLTSPEGLSGEQKSQWLSTIKAVVQSAKYWNLAECTFEASGEGVIMKKRQITPDVYKVTPVMNTHPYQSEAVSDVWSLSKTSMTFQPKKASLQPLTISLDELFSSRGEFISVGGNGRMSHKEAILLGLRYKKLYNQARVKYSL

SEQ ID NO: 69 - protein, 265 aa, (Artificial Sequence)
MDNLTKVREYLKSYSRLDQAVGEIDEIEAQRAEKSNYELFQEDGVEEHTKPSYFQAADDSDTESEPEIEDNQGLYAPDPEAEQVEGFIQGPLDDYADEEVDVVFTSDWKQPELESDEHGKTLRLTSPEGLSGEQKSQWLSTIKAVVQSAKYWNLAECTFEASGEGVIMKERQITPDVYKVTPVMNTHPYQSEAVSDVWSLSKTSMTFQPKKASLQPLTISLDELFSSRGEFISVGGNGRMSHKEAILLGLRYKKLYNQARVKYSL

SEQ ID NO: 70 - protein, 265 aa, (Artificial Sequence)
MDNLTKVREYLKSYSRLDQAVGEIDEIEAQRAEKSNYELFQEDGVEEHTKPSYFQAADDSDTESEPEIEDNQGLYAPDPEAEQVEGFIQGPLDDYADEEVDVVFTSDWKQPELESDEHGKTLRLTSPEGLSGEQKSQWLSTIKAVVQSAKYWNLAECTFEASGEGVIMKERQITPDVYKVTPVMNTHPSQSEAVSDVWSLSKTSMTFQPKKASLQPLTISLDELFSSRGEFISVGGNGRMSHKEAILLGLRYKKLYNQARVKYSL

SEQ ID NO: 71 - protein, 265 aa, (Artificial Sequence)
MDNLTKVREYLKSYSRLDQAVGEIDEIEAQRAEKSNYELFQEDGVEEHTKPSYFQAADDSDTESEPEIEDNQGLYAPDPEAEQVEGFIQGPLDDYADEEVDVVFTSDWKQPELESDEHGKTLRLTSPEGLSGEQKSQWLSTIKAVVQSAKYWNLAECTFEASGEGVIMKERQITPDVYKVTPVMNTHPSQSEAVSDVWSLSKTSMTFQPKKASLQPLTISLDELFSSRGEFISVGGDGRMSHKEAILLGLRYKKLYNQARVKYSL

SEQ ID NO: 72 - protein, 264 aa, (Artificial Sequence)
DNLTKVREYLKSYSRLDQAVGEIDEIEAQRAEKSNYELFQEDGVEEHTRPSYFQAADDSDTESEPEIEDNQGLYAPDPEAEQVEGFIQGPLDDYADEEVDVVFTSDWKQPELESDEHGKTLRLTSPEGLSGEQKSQWLSTIKAVVQSAKYWNLAECTFEASGEGVIMKERQITPDVYKVTPVMNTHPSQSEAVSDVWSLSKTSMTFQPKKASLQPLTISLDELFSSRGEFISVGGDGRMSHKEAILLGLRYKKLYNQARVKYSL

SEQ ID NO: 73 - protein, 265 aa, (Artificial Sequence)
MDNLTKVREYLKSYSRLDQAVGEIDEIEAQRAEKSNYELFQEDGVEEHTRPSYFQAADDSDTESEPEIEDNQGLYVPDPEAEQVEGFIQGPLDDYADEEVDVVFTSDWKQPELESDEHGKTLRLTSPEGLSGEQKSQWLSTIKAVVQSAKYWNLAECTFEASGEGVIMKERQITPDVYKVTPVMNTHPSQSEAVSDVWSLSKTSMTFQPKKASLQPLTISLDELFSSRGEFISVGGDGRMSHKEAILLGLRYKKLYNQARVKYSL

SEQ ID NO: 74 - protein, 265 aa, (Artificial Sequence)
MDNLTKVREYLKSYSRLDQAVGEIDEIEAQRAEKSNYELFQEDGVEEHTRPSYFQAADDSDTESEPEIEDNQGLYVPDPEAEQVEGFIQGPLDDYADEDVDVVFTSDWKQPELESDEHGKTLRLTSPEGLSGEQKSQWLSTIKAVVQSAKYWNLAECTFEASGEGVIMKERQITPDVYKVTPVMNTHPSQSEAVSDVWSLSKTSMTFQPKKASLQPLTISLDELFSSRGEFISVGGDGRMSHKEAILLGLRYKKLYNQARVKYSL

SEQ ID NO: 75 - protein, 265 aa, (Artificial Sequence)
MDNLTKVREYLKSYSRLDQAVGEIDEIEAQRAEKSNYELFQEDGVEEHTRPSYFQAADDSDTESEPEIEDNQGLYVPDPEAEQVEGFIQGPLDDYADEDVDVVFTSDWKQPELESDEHGKTLRLTLPEGLSGEQKSQWLSTIKAVVQSAKYWNLAECTFEASGEGVIMKERQITPDVYKVTPVMNTHPSQSEAVSDVWSLSKTSMTFQPKKASLQPLTISLDELFSSRGEFISVGGDGRMSHKEAILLGLRYKKLYNQARVKYSL

SEQ ID NO: 76 - protein, 265 aa, (Artificial Sequence)
MDNLTKVREYLKSYSRLDQAVGEIDEIEAQRAEKSNYELFQEDGVEEHTRPSYFQAADDSDTESEPEIEDNQGLYVPDPEAEQVEGFIQGPLDDYADEDVDVVFTSDWKQPELESDEHGKTLRLTLPEGLSGEQKSQWLLTIKAVVQSAKYWNLAECTFEASGEGVIMKERQITPDVYKVTPVMNTHPSQSEAVSDVWSLSKTSMTFQPKKASLQPLTISLDELFSSRGEFISVGGDGRMSHKEAILLGLRYKKLYNQARVKYSL

SEQ ID NO: 77 - protein, 265 aa, (Artificial Sequence)
MDNLTKVREYLKSYSRLDQAVGEIDEIEAQRAEKSNYELFQEDGVEEHTRPSYFQAADDSDTESEPEIEDNQGLYVPDPEAEQVEGFIQGPLDDYADEDVDVVFTSDWKQPELESDEHGKTLRLTLPEGLSGEQKSQWLLTIKAVVQSAKHWNLAECTFEASGEGVIMKERQITPDVYKVTPVMNTHPSQSEAVSDVWSLSKTSMTFQPKKASLQPLTISLDELFSSRGEFISVGGDGRMSHKEAILLGLRYKKLYNQARVKYSL

SEQ ID NO: 78 - protein, 265 aa, (Artificial Sequence)
MDNLTKVREYLKSYSRLDQAVGEIDEIEAQRAEKSNYELFQEDGVEEHTRPSYFQAADDSDTESEPEIEDNQGLYVPDPEAEQVEGFIQGPLDDYADEDVDVVFTSDWKQPELESDEHGKTLRLTLPEGLSGEQKSQWLLTIKAVVQSAKHWNLAECTFEASGEGVIIKERQITPDVYKVTPVMNTHPSQSEAVSDVWSLSKTSMTFQPKKASLQPLTISLDELFSSRGEFISVGGDGRMSHKEAILLGLRYKKLYNQARVKYSL

SEQ ID NO: 79 - protein, 265 aa, (Artificial Sequence)
MDNLTKVREYLKSYSRLDQAVGEIDEIEAQRAEKSNYELFQEDGVEEHTRPSYFQAADDSDTESEPEIEDNQGLYVPDPEAEQVEGFIQGPLDDYADEDVDVVFTSDWKQPELESDEHGKTLRLTLPEGLSGEQKSQWLLTIKAVVQSAKHWNLAECTFEASGEGVIIKKRQITPDVYKVTPVMNTHPSQSEAVSDVWSLSKTSMTFQPKKASLQPLTISLDELFSSRGEFISVGGDGRMSHKEAILLGLRYKKLYNQARVKYSL

SEQ ID NO: 80 - protein, 265 aa, (Artificial Sequence)
MDNLTKVREYLKSYSRLDQAVGEIDEIEAQRAEKSNYELFQEDGVEEHTRPSYFQAADDSDTESEPEIEDNQGLYVPDPEAEQVEGFIQGPLDDYADEDVDVVFTSDWKQPELESDEHGKTLRLTLPEGLSGEQKSQWLLTIKAVVQSAKHWNLAECTFEASGEGVIIKKRQITPDVYKVTPVMNTHPYQSEAVSDVWSLSKTSMTFQPKKASLQPLTISLDELFSSRGEFISVGGDGRMSHKEAILLGLRYKKLYNQARVKYSL

SEQ ID NO: 81 - protein, 2109 aa, Vesicular Stomatitis Virus
MEVHDFETDEFNDFNEDDYATREFLNPDERMTYLNHADYNLNSPLISDDIDNLIRKFNSLPIPSMWDSKNWDGVLEMLTSCQANPISTSQMHKWMGSWLMSDNHDASQGYSFLHEVDKEAEITFDVVETFIRGWGNKPIEYIKKERWTDSFKILAYLCQKFLDLHKLTLILNAVSEVELLNLARTFKGKVRRSSHGTNICRIRVPSLGPTFISEGWAYFKKLDILMDRNFLLMVKDVIIGRMQTVLSMVCRIDNLFSEQDIFSLLNIYRIGDKIVERQGNFSYDLIKMVEPICNLKLMKLARESRPLVPQFPHFENHIKTSVDEGAKIDRGIRFLHDQIMSVKTVDLTLVIYGSFRHWGHPFIDYYTGLEKLHSQVTMKKDIDVSYAKALASDLARIVLFQQFNDHKKWFVNGDLLPHDHPFKSHVKENTWPTAAQVQDFGDKWHELPLIKCFEIPDLLDPSIIYSDKSHSMNRSEVLKHVRMNPNIPIPSKKVLQTMLDTKATNWKEFLKEIDEKGLDDDDLIIGLKGKERELKLAGRFFSLMSWKLREYFVITEYLIKTHFVPMFKGLTMADDLTAVIKKMLDSSSGQGLKSYEAICIANHIDYEKWNNHQRKLSNGPVFRVMGQFLGYPSLIERTHEFFEKSLIYYNGRPDLMRVHNNTLINSTSQRVCWQGQEGGLEGLRQKGWSILNLLVIQREAKIRNTAVKVLAQGDNQVICTQYKTKKSRNVVELQGALNQMVSNNEKIMTAIKIGTGKLGLLINDDETMQSADYLNYGKIPIFRGVIRGLETKRWSRVTCVTNDQIPTCANIMSSVSTNALTVAHFAENPINAMIQYNYFGTFARLLLMMHDPALRQSLYEVQDKIPGLHSSTFKYAMLYLDPSIGGVSGMSLSRFLIRAFPDPVTESLSFWRFIHVHARSEHLKEMSAVFGNPEIAKFRITHIDKLVEDPTSLNIAMGMSPANLLKTEVKKCLIESRQTIRNQVIKDATIYLYHEEDRLRSFLWSINPLFPRFLSEFKSGTFLGVADGLISLFQNSRTIRNSFKKKYHRELDDLIVRSEVSSLTHLGKLHLRRGSCKMWTCSATHADTLRYKSWGRTVIGTTVPHPLEMLGPQHRKETPCAPCNTSGFNYVSVHCPDGIHDVFSSRGPLPAYLGSKTSESTSILQPWERESKVPLIKRATRLRDAISWFVEPDSKLAMTILSNIHSLTGEEWTKRQHGFKRTGSALHRFSTSRMSHGGFASQSTAALTRLMATTDTMRDLGDQNFDFLFQATLLYAQITTTVARDGWITSCTDHYHIACKSCLRPIEEITLDSSMDYTPPDVSHVLKTWRNGEGSWGQEIKQIYPLEGNWKNLAPAEQSYQVGRCIGFLYGDLAYRKSTHAEDSSLFPLSIQGRIRGRGFLKGLLDGLMRASCCQVIHRRSLAHLKRPANAVYGGLIYLIDKLSVSPPFLSLTRSGPIRDELETIPHKIPTSYPTSNRDMGVIVRNYFKYQCRLIEKGKYRSHYSQLWLFSDVLSIDFIGPFSISTTLLQILYKPFLSGKDKNELRELANLSSLLRSGEGWEDIHVKFFTKDILLCPEEIRHACKFGIAKDNNKDMSYPPWGRESRGTITTIPVYYTTTPYPKMLEMPPRIQNPLLSGIRLGQLPTGAHYKIRSILHGMGIHYRDFLSCGDGSGGMTAALLRENVHSRGIFNSLLELSGSVMRGASPEPPSALETLGGDKSRCVNGETCWEYPSDLCDPRTWDYFLRLKAGLGLQIDLIVMDMEVRDSSTSLKIETNVRNYVHRILDEQGVLIYKTYGTYICESEKNAVTILGPMFKTVDLVQTEFSSSQTSEVYMVCKGLKKLIDEPNPDWSSINESWKNLYAFQSSEQEFARAKKVSTYFTLTGIPSQFIPDPFVNIETMLQIFGVPTGVSHAAALKSSDRPADLLTISLFYMAIISYYNINHIRVGPIPPNPPSDGIAQNVGIAITGISFWLSLMEKDIPLYQQCLAVIQQSFPIRWEAVSVKGGYKQKWSTRGDGLPKDTRISDSLAPIGNWIRSLELVRNQVRLNPFNEILFNQLCRTVDNHLKWSNLRRNTGMIEWINRRISKEDRSILMLKSDLHEENSWRD

SEQ ID NO: 82 - protein, 2109 aa, (Artificial Sequence)
MEVHDFETDEFNDFNEDDYATREFLNPDERMTYLNHADYNLNSPLISDDIDNLIRKFNSLPIPSMWDSKNWDGVLEMLTSCQANPIPTSQMHKWMGSWLMSDNHDASQGYSFLHEVDKEAEITFDVVETFIRGWGNKPIEYIKKERWTDSFKILAYLCQKFLDLHKLTLILNAVSEVELLNLARTFKGKVRRSSHGTNICRIRVPSLGPTFISEGWAYFKKLDILMDRNFLLMVKDVIIGRMQTVLSMVCRIDNLFSEQDIFSLLNIYRIGDKIVERQGNFSYDLIKMVEPICNLKLMKLARESRPLVPQFPHFENHIKTSVDEGAKIDRGIRFLHDQIMSVKTVDLTLVIYGSFRHWGHPFIDYYTGLEKLHSQVTMKKDIDVSYAKALASDLARIVLFQQFNDHKKWFVNGDLLPHDHPFKSHVKENTWPTAAQVQDFGDKWHELPLIKCFEIPDLLDPSIIYSDKSHSMNRSEVLKHVRMNPNIPIPSKKVLQTMLDTKATNWKEFLKEIDEKGLDDDDLIIGLKGKERELKLAGRFFSLMSWKLREYFVITEYLIKTHFVPMFKGLTMADDLTAVIKKMLDSSSGQGLKSYEAICIANHIDYEKWNNHQRKLSNGPVFRVMGQFLGYPSLIERTHEFFEKSLIYYNGRPDLMRVHNNTLINSTSQRVCWQGQEGGLEGLRQKGWSILNLLVIQREAKIRNTAVKVLAQGDNQVICTQYKTKKSRNVVELQGALNQMVSNNEKIMTAIKIGTGKLGLLINDDETMQSADYLNYGKIPIFRGVIRGLETKRWSRVTCVTNDQIPTCANIMSSVSTNALTVAHFAENPINAMIQYNYFGTFARLLLMMHDPALRQSLYEVQDKIPGLHSSTFKYAMLYLDPSIGGVSGMSLSRFLIRAFPDPVTESLSFWRFIHVHARSEHLKEMSAVFGNPEIAKFRITHIDKLVEDPTSLNIAMGMSPANLLKTEVKKCLIESRQTIRNQVIKDATIYLYHEEDRLRSFLWSINPLFPRFLSEFKSGTFLGVADGLISLFQNSRTIRNSFKKKYHRELDDLIVRSEVSSLTHLGKLHLRRGSCKMWTCSATHADTLRYKSWGRTVIGTTVPHPLEMLGPQHRKETPCAPCNTSGFNYVSVHCPDGIHDVFSSRGPLPAYLGSKTSESTSILQPWERESKVPLIKRATRLRDAISWFVEPDSKLAMTILSNIHSLTGEEWTKRQHGFKRTGSALHRFSTSRMSHGGFASQSTAALTRLMATTDTMRDLGDQNFDFLFQATLLYAQITTTVARDGWITSCTDHYHIACKSCLRPIEEITLDSSMDYTPPDVSHVLKTWRNGEGSWGQEIKQIYPLEGNWKNLAPAEQSYQVGRCIGFLYGDLAYRKSTHAEDSSLFPLSIQGRIRGRGFLKGLLDGLMRASCCQVIHRRSLAHLKRPANAVYGGLIYLIDKLSVSPPFLSLTRSGPIRDELETIPHKIPTSYPTSNRDMGVIVRNYFKYQCRLIEKGKYRSHYSQLWLFSDVLSIDFIGPFSISTTLLQILYKPFLSGKDKNELRELANLSSLLRSGEGWEDIHVKFFTKDILLCPEEIRHACKFGIAKDNNKDMSYPPWGRESRGTITTIPVYYTTTPYPKMLEMPPRIQNPLLSGIRLGQLPTGAHYKIRSILHGMGIHYRDFLSCGDGSGGMTAALLRENVHSRGIFNSLLELSGSVMRGASPEPPSALETLGGDKSRCVNGETCWEYPSDLCDPRTWDYFLRLKAGLGLQIDLIVMDMEVRDSSTSLKIETNVRNYVHRILDEQGVLIYKTYGTYICESEKNAVTILGPMFKTVDLVQTEFSSSQTSEVYMVCKGLKKLIDEPNPDWSSINESWKNLYAFQSSEQEFARAKKVSTYFTLTGIPSQFIPDPFVNIETMLQIFGVPTGVSHAAALKSSDRPADLLTISLFYMAIISYYNINHIRVGPIPPNPPSDGIAQNVGIAITGISFWLSLMEKDIPLYQQCLAVIQQSFPIRWEAVSVKGGYKQKWSTRGDGLPKDTRISDSLAPIGNWIRSLELVRNQVRLNPFNEILFNQLCRTVDNHLKWSNLRRNTGMIEWINRRISKEDRSILMLKSDLHEENSWRD

SEQ ID NO: 83 - protein, 2109 aa, (Artificial Sequence)
MEVHDFETDEFNDFNEDDYATREFLNPDERMTYLNHADYNLNSPLISDDIDNLIRKFNSLPIPSMWDSKNWDGVLEMLTSCQANPIPTSQMHKWMGSWLMSDNHDASQGYSFLHEVDKEAEITFDVVETFIRGWGNKPIEYIKKERWTDSFKILAYLCQKFLDLHKLTLILNAVSEVELLNLARTFKGKVRRSSHGTNICRIRVPSLGPTFISEGWAYFKKLDILMDRNFLLMVKDVIIGRMQTVLSMVCRIDNLFSEQDIFSLLNIYRIGDKIVERQGNFSYDLIKMVEPICNLKLMKLARESRPLVPQFPHFENHIKTSVDEGAKIDRGIRFLHDQIMSVKTVDLTLVIYGSFRHWGHPFIDYYTGLEKLHSQVTMKKDIDVSYAKALASDLARIVLFQQFNDHKKWFVNGDLLPHDHPFKSHVKENTWPTAAQVQDFGDKWHELPLIKCFEIPDLLDPSIIYSDKSHSMNRSEVLKHVRMNPNTPIPSKKVLQTMLDTKATNWKEFLKEIDEKGLDDDDLIIGLKGKERELKLAGRFFSLMSWKLREYFVITEYLIKTHFVPMFKGLTMADDLTAVIKKMLDSSSGQGLKSYEAICIANHIDYEKWNNHQRKLSNGPVFRVMGQFLGYPSLIERTHEFFEKSLIYYNGRPDLMRVHNNTLINSTSQRVCWQGQEGGLEGLRQKGWSILNLLVIQREAKIRNTAVKVLAQGDNQVICTQYKTKKSRNVVELQGALNQMVSNNEKIMTAIKIGTGKLGLLINDDETMQSADYLNYGKIPIFRGVIRGLETKRWSRVTCVTNDQIPTCANIMSSVSTNALTVAHFAENPINAMIQYNYFGTFARLLLMMHDPALRQSLYEVQDKIPGLHSSTFKYAMLYLDPSIGGVSGMSLSRFLIRAFPDPVTESLSFWRFIHVHARSEHLKEMSAVFGNPEIAKFRITHIDKLVEDPTSLNIAMGMSPANLLKTEVKKCLIESRQTIRNQVIKDATIYLYHEEDRLRSFLWSINPLFPRFLSEFKSGTFLGVADGLISLFQNSRTIRNSFKKKYHRELDDLIVRSEVSSLTHLGKLHLRRGSCKMWTCSATHADTLRYKSWGRTVIGTTVPHPLEMLGPQHRKETPCAPCNTSGFNYVSVHCPDGIHDVFSSRGPLPAYLGSKTSESTSILQPWERESKVPLIKRATRLRDAISWFVEPDSKLAMTILSNIHSLTGEEWTKRQHGFKRTGSALHRFSTSRMSHGGFASQSTAALTRLMATTDTMRDLGDQNFDFLFQATLLYAQITTTVARDGWITSCTDHYHIACKSCLRPIEEITLDSSMDYTPPDVSHVLKTWRNGEGSWGQEIKQIYPLEGNWKNLAPAEQSYQVGRCIGFLYGDLAYRKSTHAEDSSLFPLSIQGRIRGRGFLKGLLDGLMRASCCQVIHRRSLAHLKRPANAVYGGLIYLIDKLSVSPPFLSLTRSGPIRDELETIPHKIPTSYPTSNRDMGVIVRNYFKYQCRLIEKGKYRSHYSQLWLFSDVLSIDFIGPFSISTTLLQILYKPFLSGKDKNELRELANLSSLLRSGEGWEDIHVKFFTKDILLCPEEIRHACKFGIAKDNNKDMSYPPWGRESRGTITTIPVYYTTTPYPKMLEMPPRIQNPLLSGIRLGQLPTGAHYKIRSILHGMGIHYRDFLSCGDGSGGMTAALLRENVHSRGIFNSLLELSGSVMRGASPEPPSALETLGGDKSRCVNGETCWEYPSDLCDPRTWDYFLRLKAGLGLQIDLIVMDMEVRDSSTSLKIETNVRNYVHRILDEQGVLIYKTYGTYICESEKNAVTILGPMFKTVDLVQTEFSSSQTSEVYMVCKGLKKLIDEPNPDWSSINESWKNLYAFQSSEQEFARAKKVSTYFTLTGIPSQFIPDPFVNIETMLQIFGVPTGVSHAAALKSSDRPADLLTISLFYMAIISYYNINHIRVGPIPPNPPSDGIAQNVGIAITGISFWLSLMEKDIPLYQQCLAVIQQSFPIRWEAVSVKGGYKQKWSTRGDGLPKDTRISDSLAPIGNWIRSLELVRNQVRLNPFNEILFNQLCRTVDNHLKWSNLRRNTGMIEWINRRISKEDRSILMLKSDLHEENSWRD

SEQ ID NO: 84 - protein, 2109 aa, (Artificial Sequence)
MEVHDFETDEFNDFNEDDYATREFLNPDERMTYLNHADYNLNSPLISDDIDNLIRKFNSLPIPSMWDSKNWDGVLEMLTSCQANPISTSQMHKWMGSWLMSDNHDASQGYSFLHEVDKEAEITFDVVETFIRGWGNKPIEYIKKERWTDSFKILAYLCQKFLDLHKLTLILNAVSEVELLNLARTFKGKVRRSSHGTNICRIRVPSLGPTFISEGWAYFKKLDILMDRNFLLMVKDVIIGRMQTVLSMVCRIDNLFSEQDIFSLLNIYRIGDKIVERQGNFSYDLIKMVEPICNLKLMKLARESRPLVPQFPHFENHIKTSVDEGAKIDRGIRFLHDQIMSVKTVDLTLVIYGSFRHWGHPFIDYYTGLEKLHSQVTMKKDIDVSYAKALASDLARIVLFQQFNDHKKWFVNGDLLPHDHPFKSHVKENTWPTAAQVQDFGDKWHELPLIKCFEIPDLLDPSIIYSDKSHSMNRSEVLKHVRMNPNTPIPSKKVLQTMLDTKATNWKEFLKEIDEKGLDDDDLIIGLKGKERELKLAGRFFSLMSWKLREYFVITEYLIKTHFVPMFKGLTMADDLTAVIKKMLDSSSGQGLKSYEAICIANHIDYEKWNNHQRKLSNGPVFRVMGQFLGYPSLIERTHEFFEKSLIYYNGRPDLMRVHNNTLINSTSQRVCWQGQEGGLEGLRQKGWSILNLLVIQREAKIRNTAVKVLAQGDNQVICTQYKTKKSRNVVELQGALNQMVSNNEKIMTAIKIGTGKLGLLINDDETMQSADYLNYGKIPIFRGVIRGLETKRWSRVTCVTNDQIPTCANIMSSVSTNALTVAHFAENPINAMIQYNYFGTFARLLLMMHDPALRQSLYEVQDKIPGLHSSTFKYAMLYLDPSIGGVSGMSLSRFLIRAFPDPVTESLSFWRFIHVHARSEHLKEMSAVFGNPEIAKFRITHIDKLVEDPTSLNIAMGMSPANLLKTEVKKCLIESRQTIRNQVIKDATIYLYHEEDRLRSFLWSINPLFPRFLSEFKSGTFLGVADGLISLFQNSRTIRNSFKKKYHRELDDLIVRSEVSSLTHLGKLHLRRGSCKMWTCSATHADTLRYKSWGRTVIGTTVPHPLEMLGPQHRKETPCAPCNTSGFNYVSVHCPDGIHDVFSSRGPLPAYLGSKTSESTSILQPWERESKVPLIKRATRLRDAISWFVEPDSKLAMTILSNIHSLTGEEWTKRQHGFKRTGSALHRFSTSRMSHGGFASQSTAALTRLMATTDTMRDLGDQNFDFLFQATLLYAQITTTVARDGWITSCTDHYHIACKSCLRPIEEITLDSSMDYTPPDVSHVLKTWRNGEGSWGQEIKQIYPLEGNWKNLAPAEQSYQVGRCIGFLYGDLAYRKSTHAEDSSLFPLSIQGRIRGRGFLKGLLDGLMRASCCQVIHRRSLAHLKRPANAVYGGLIYLIDKLSVSPPFLSLTRSGPIRDELETIPHKIPTSYPTSNRDMGVIVRNYFKYQCRLIEKGKYRSHYSQLWLFSDVLSIDFIGPFSISTTLLQILYKPFLSGKDKNELRELANLSSLLRSGEGWEDIHVKFFTKDILLCPEEIRHACKFGIAKDNNKDMSYPPWGRESRGTITTIPVYYTTTPYPKMLEMPPRIQNPLLSGIRLGQLPTGAHYKIRSILHGMGIHYRDFLSCGDGSGGMTAALLRENVHSRGIFNSLLELSGSVMRGASPEPPSALETLGGDKSRCVNGETCWEYPSDLCDPRTWDYFLRLKAGLGLQIDLIVMDMEVRDSSTSLKIETNVRNYVHRILDEQGVLIYKTYGTYICESEKNAVTILGPMFKTVDLVQTEFSSSQTSEVYMVCKGLKKLIDEPNPDWSSINESWKNLYAFQSSEQEFARAKKVSTYFTLTGIPSQFIPDPFVNIETMLQIFGVPTGVSHAAALKSSDRPADLLTISLFYMAIISYYNINHIRVGPIPPNPPSDGIAQNVGIAITGISFWLSLMEKDIPLYQQCLAVIQQSFPIRWEAVSVKGGYKQKWSTRGDGLPKDTRISDSLAPIGNWIRSLELVRNQVRLNPFNEILFNQLCRTVDNHLKWSNLRRNTGMIEWINRRISKEDRSILMLKSDLHEENSWRD